European Patent Specification EP 3 775 193 B1, published September 17, 2025. Title: PEPTIDES AND CONJUGATES. Applicant: The University of Liverpool. The sequence listing filed with the application follows.

SEQUENCE LISTING (38 sequences)

SEQ ID NO: 1 - protein, 660 aa, Homo sapiens
MEALMARGALTGPLRALCLLGCLLSHAAAAPSPIIKFPGDVAPKTDKELAVQYLNTFYGCPKESCNLFVLKDTLKKMQKFFGLPQTGDLDQNTIETMRKPRCGNPDVANYNFFPRKPKWDKNQITYRIIGYTPDLDPETVDDAFARAFQVWSDVTPLRFSRIHDGEADIMINFGRWEHGDGYPFDGKDGLLAHAFAPGTGVGGDSHFDDDELWTLGEGQVVRVKYGNADGEYCKFPFLFNGKEYNSCTDTGRSDGFLWCSTTYNFEKDGKYGFCPHEALFTMGGNAEGQPCKFPFRFQGTSYDSCTTEGRTDGYRWCGTTEDYDRDKKYGFCPETAMSTVGGNSEGAPCVFPFTFLGNKYESCTSAGRSDGKMWCATTANYDDDRKWGFCPDQGYSLFLVAAHEFGHAMGLEHSQDPGALMAPIYTYTKNFRLSQDDIKGIQELYGASPDIDLGTGPTPTLGPVTPEICKQDIVFDGIAQIRGEIFFFKDRFIWRTVTPRDKPMGPLLVATFWPELPEKIDAVYEAPQEEKAVFFAGNEYWIYSASTLERGYPKPLTSLGLPPDVQRVDAAFNWSKNKKTYIFAGDKFWRYNEVKKKMDPGFPKLIADAWNAIPDNLDAVVDLQGGGHSYFFKGAYYLKLENQSLKSVKFGSIKSDWLGC

SEQ ID NO: 2 - protein, 165 aa, Homo sapiens
ADGEYCKFPFLFNGKEYNSCTDTGRSDGFLWCSTTYNFEKDGKYGFCPHEALFTMGGNAEGQPCKFPFRFQGTSYDSCTTEGRTDGYRWCGTTEDYDRDKKYGFCPETAMSTVGGNSEGAPCVFPFTFLGNKYESCTSAGRSDGKMWCATTANYDDDRKWGFCPD

SEQ ID NO: 3 - protein, 175 aa, Artificial Sequence
  Amino acid sequence of peptide comprising the CBD of MMP-2 with additional residues added
RVKYGNADGEYCKFPFLFNGKEYNSCTDTGRSDGFLWCSTTYNFEKDGKYGFCPHEALFTMGGNAEGQPCKFPFRFQGTSYDSCTTEGRTDGYRWCGTTEDYDRDKKYGFCPETAMSTVGGNSEGAPCVFPFTFLGNKYESCTSAGRSDGKMWCATTANYDDDRKWGFCPDQGYS

SEQ ID NO: 4 - DNA, 525 bp, Homo sapiens
cgtgtgaaatatggtaatgccgatggcgaatattgcaaatttccgtttctgtttaacggcaaagagtataatagctgtaccgataccggtcgtagtgatggttttctgtggtgtagcaccacctataactttgagaaagatggcaaatatggcttttgtccgcatgaagcactgtttaccatgggtggtaatgcggaaggtcagccgtgtaaatttccttttcgctttcagggcaccagctatgatagttgtaccaccgaaggtcgtaccgatggttatcgttggtgcggtacaaccgaagattatgatcgtgacaaaaaatacggtttctgtccggaaaccgcaatgagcaccgttggtggtaatagtgaaggtgcaccgtgtgtttttccgtttacctttctgggtaacaaatatgaaagctgtaccagtgcaggtcgttcagatggtaaaatgtggtgcgcaaccaccgcaaattatgatgatgatcgtaaatggggtttttgcccagatcagggttatagc

SEQ ID NO: 5 - DNA, 528 bp, Artificial Sequence
  DNA sequence encoding the CBD of MMP-2 (with stop codon)
cgtgtgaaatatggtaatgccgatggcgaatattgcaaatttccgtttctgtttaacggcaaagagtataatagctgtaccgataccggtcgtagtgatggttttctgtggtgtagcaccacctataactttgagaaagatggcaaatatggcttttgtccgcatgaagcactgtttaccatgggtggtaatgcggaaggtcagccgtgtaaatttccttttcgctttcagggcaccagctatgatagttgtaccaccgaaggtcgtaccgatggttatcgttggtgcggtacaaccgaagattatgatcgtgacaaaaaatacggtttctgtccggaaaccgcaatgagcaccgttggtggtaatagtgaaggtgcaccgtgtgtttttccgtttacctttctgggtaacaaatatgaaagctgtaccagtgcaggtcgttcagatggtaaaatgtggtgcgcaaccaccgcaaattatgatgatgatcgtaaatggggtttttgcccagatcagggttatagctaa

SEQ ID NO: 6 - protein, 49 aa, Homo sapiens
ADGEYCKFPFLFNGKEYNSCTDTGRSDGFLWCSTTYNFEKDGKYGFCPH

SEQ ID NO: 7 - protein, 60 aa, Artificial Sequence
  Amino acid sequence comprising module 1 of the CBD of MMP-2 with additional residues
VKYGNADGEYCKFPFLFNGKEYNSCTDTGRSDGFLWCSTTYNFEKDGKYGFCPHEALFTM

SEQ ID NO: 8 - protein, 55 aa, Artificial Sequence
  a variant module corresponding to module 1 of the CBD of MMP-2
VRVKYVNADGEYCKFPFLFNGKEYNSCTDTGRSDGFLWCSTTYNFEKDGKYGFCP

SEQ ID NO: 9 - DNA, 180 bp, Homo sapiens
gtgaaatatggtaatgccgatggcgaatattgcaaatttccgtttctgtttaacggcaaagagtataatagctgtaccgataccggtcgtagtgatggttttctgtggtgtagcaccacctataactttgagaaagatggcaaatatggcttttgtccgcatgaagcactgtttaccatg

SEQ ID NO: 10 - DNA, 183 bp, Artificial Sequence
  DNA sequence encoding an amino acid sequence comprising module 1 of the CBD of MMP-2 with stop codon
gtgaaatatggtaatgccgatggcgaatattgcaaatttccgtttctgtttaacggcaaagagtataatagctgtaccgataccggtcgtagtgatggttttctgtggtgtagcaccacctataactttgagaaagatggcaaatatggcttttgtccgcatgaagcactgtttaccatgtaa

SEQ ID NO: 11 - protein, 49 aa, Homo sapiens
AEGQPCKFPFRFQGTSYDSCTTEGRTDGYRWCGTTEDYDRDKKYGFCPE

SEQ ID NO: 12 - protein, 59 aa, Artificial Sequence
  Amino acid sequence comprising module 2 of the CBD of MMP-2 with additional residues
ALFTMGGNAEGQPCKFPFRFQGTSYDSCTTEGRTDGYRWCGTTEDYDRDKKYGFCPETA

SEQ ID NO: 13 - protein, 55 aa, Homo sapiens
VFTMYGNAEGQPCKFPFRFQGTSYDSCTTEGRTDGYRWCGTTEDYDRDKKYGFCP

SEQ ID NO: 14 - protein, 55 aa, Artificial Sequence
  Amino acid sequence of a variant module corresponding to module 2 of the CBD of MMP-2
LFTMGGNAEGQPCKFPFRFQGTSYDSCTTEGRTDGYRWCGTTEDYDRDKKYGFCP

SEQ ID NO: 15 - DNA, 177 bp, Artificial Sequence
  DNA sequence encoding a peptide comprising a variant module corresponding to module 2 of the CBD of MMP-2
gcactgtttaccatgggtggtaatgcggaaggtcagccgtgtaaatttccttttcgctttcagggcaccagctatgatagttgtaccaccgaaggtcgtaccgatggttatcgttggtgcggtacaaccgaagattatgatcgtgacaaaaaatacggtttctgtccggaaaccgca

SEQ ID NO: 16 - DNA, 180 bp, Artificial Sequence
  DNA sequence encoding a peptide comprising a module corresponding to module 2 of the CBD of MMP-2 with stop codon
gcactgtttaccatgggtggtaatgcggaaggtcagccgtgtaaatttccttttcgctttcagggcaccagctatgatagttgtaccaccgaaggtcgtaccgatggttatcgttggtgcggtacaaccgaagattatgatcgtgacaaaaaatacggtttctgtccggaaaccgcataa

SEQ ID NO: 17 - protein, 49 aa, Homo sapiens
SEGAPCVFPFTFLGNKYESCTSAGRSDGKMWCATTANYDDDRKWGFCPD

SEQ ID NO: 18 - protein, 58 aa, Artificial Sequence
  Amino acid sequence of a peptide comprising module 3 of the CBD of MMP-2 with additional residues
MSTVGGNSEGAPCVFPFTFLGNKYESCTSAGRSDGKMWCATTANYDDDRKWGFCPDQG

SEQ ID NO: 19 - protein, 55 aa, Artificial Sequence
  Amino acid sequence of a variant module corresponding to module 3 of the CBD of MMP-2
MSTVGGNSEGAPCVFPFTFLGNKYESCTSAGRSDGKMWCATTANYDDDRKWGFCP

SEQ ID NO: 20 - DNA, 174 bp, Homo sapiens
atgagcaccgttggtggtaatagtgaaggtgcaccgtgtgtttttccgtttacctttctgggtaacaaatatgaaagctgtaccagtgcaggtcgttcagatggtaaaatgtggtgcgcaaccaccgcaaattatgatgatgatcgtaaatggggtttttgcccagatcagggt

SEQ ID NO: 21 - DNA, 177 bp, Artificial Sequence
  DNA encoding a peptide comprising a module corresponding to module 3 of the CBD of MMP-2 with stop codon
atgagcaccgttggtggtaatagtgaaggtgcaccgtgtgtttttccgtttacctttctgggtaacaaatatgaaagctgtaccagtgcaggtcgttcagatggtaaaatgtggtgcgcaaccaccgcaaattatgatgatgatcgtaaatggggtttttgcccagatcagggttaa

SEQ ID NO: 22 - protein, 181 aa, Artificial Sequence
  Exemplary peptide 111 comprising three modules corresponding to module 1 of the CBD of MMP-2
EGQVVRVKYGNADGEYCKFPFLFNGKEYNSCTDTGRSDGFLWCSTTYNFEKDGKYGFCPHEALFVMYGNADGEYCKFPFLFNGKEYNSCTDTGRSDGFRWCSTTYNFEKDGKYGFCPETAVRVKYGNADGEYCKFPFLFNGKEYNSCTDTGRSDGFLWCSTTYNFEKDGKYGFCPDQGYSL

SEQ ID NO: 23 - DNA, 543 bp, Artificial Sequence
  DNA sequence encoding exemplary peptide 111
gaaggtcaggttgttcgtgtgaaatatggtaatgcagatggcgagtattgcaaatttccgtttctgtttaacggcaaagagtataatagctgtaccgataccggtcgtagtgatggttttctgtggtgtagcaccacctataactttgagaaagatggcaaatatggcttttgtccgcatgaagcactgtttgtgatgtatggcaatgccgatggtgaatactgtaaattcccatttctgttcaatggtaaagaatacaactcatgcaccgatacaggccgttcagatggctttcgttggtgttcaaccacctacaatttcgaaaaagacggtaagtatggtttctgtccggaaaccgcagtgcgcgttaaatatggcaacgcggacggggaatattgtaagtttccgttcttattcaacgggaaagaatataacagttgcacagacaccggtcgctcagatggttttttatggtgctcaacaacgtataacttcgaaaaggatgggaagtacggattttgtccggatcagggttatagcctg

SEQ ID NO: 24 - DNA, 546 bp, Artificial Sequence
  DNA sequence encoding exemplary peptide 111 (with stop codon)
gaaggtcaggttgttcgtgtgaaatatgttaatgccgatggcgagtattgcaaatttccgtttctgtttaacggcaaagagtataatagctgtaccgataccggtcgtagtgatggttttctgtggtgtagcaccacctataactttgagaaagatggcaaatatggcttttgtccgcatgaagcactgtttgtgatgtatgtgaatgcggatggtgaatactgtaaattcccctttctgttcaatggtaaagaatacaactcatgcaccgatacaggccgttcagatggctttcgttggtgttcaaccacctacaatttcgaaaaagacggtaagtatggtttctgtccggaaaccgcagtgcgcgttaaatatgtgaacgcagacggggaatattgtaagtttccgttcttattcaacgggaaagaatataacagttgcacagacaccggtcgctcagatggttttttatggtgctcaacaacgtataacttcgaaaaggatgggaagtacggattttgtccggatcagggttatagcctgtaa

SEQ ID NO: 25 - protein, 181 aa, Artificial Sequence
  Exemplary peptide 222 comprising three modules corresponding to module 2 of the CBD of MMP-2
EGQVVFTMYGNAEGQPCKFPFRFQGTSYDSCTTEGRTDGYRWCGTTEDYDRDKKYGFCPHEALFTMGGNAEGQPCKFPFRFQGTSYDSCTTEGRTDGYRWCGTTEDYDRDKKYGFCPETALFTMGGNAEGQPCKFPFRFQGTSYDSCTTEGRTDGYRWCGTTEDYDRDKKYGFCPDQGYSL

SEQ ID NO: 26 - DNA, 543 bp, Artificial Sequence
  DNA sequence encoding exemplary peptide 222
gaaggtcaggttgtgtttaccatgtatggtaatgccgaaggtcagccgtgtaaatttccgtttcgttttcagggcaccagctatgatagttgtaccaccgaaggtcgtaccgatggttatcgttggtgtggtacgaccgaagattatgatcgtgataaaaagtatggcttttgtccgcatgaagccctgtttacaatgggtggcaatgcagagggccagccttgcaaattcccttttcgcttccagggtacatcttatgattcatgcacaacggaaggtcgcacagatggctaccgctggtgcggcaccacagaggattatgaccgcgacaaaaaatacggtttttgtccggaaaccgcactgttcaccatgggtggtaatgcggaaggacaaccatgcaagtttccattccgctttcagggaacctcatatgatagctgcacaacagagggacgtacggatggatacagatggtgcggtacaaccgaggactacgatagagataagaaatatggtttctgtcccgatcagggttatagcctg

SEQ ID NO: 27 - protein, 181 aa, Artificial Sequence
  Exemplary peptide 333 comprising three modules corresponding to module 3 of the CBD of MMP-2
EGQVVSTVYGNSEGAPCVFPFTFLGNKYESCTSAGRSDGFLWCATTANYDDDRKWGFCPHEALFTMGGNSEGAPCVFPFTFLGNKYESCTSAGRSDGKRWCATTANYDDDRKWGFCPETAMSTVGGNSEGAPCVFPFTFLGNKYESCTSAGRSDGKMWCATTANYDDDRKWGFCPDQGYSL

SEQ ID NO: 28 - DNA, 543 bp, Artificial Sequence
  DNA encoding exemplary peptide 333
gaaggtcaggttgttagcaccgtttatggtaatagcgaaggtgcaccgtgtgtttttccgtttacctttctgggtaacaaatatgaaagctgtaccagcgcaggtcgtagtgatggttttctgtggtgtgcaaccaccgcaaattatgatgatgatcgtaaatggggtttttgtccgcatgaagcactgtttaccatgggtggcaattctgaaggtgccccttgcgtgtttccttttacatttttaggcaacaagtacgaaagctgcacctcagccggtcgttcagatggtaaacgttggtgcgccaccacagccaactatgatgacgacagaaaatggggcttctgtcctgaaaccgcaatgagcaccgttggtggcaacagtgaaggcgctccatgcgttttcccgttcacattcctgggcaataaatacgaatcatgtacctctgcaggtcgctctgatggcaaaatgtggtgcgcgacaacggccaattacgacgatgaccgcaagtggggcttttgcccagatcagggttatagcctg

SEQ ID NO: 29 - protein, 4 aa, Artificial Sequence
  Linker sequence 1
EGQV

SEQ ID NO: 30 - protein, 58 aa, Artificial Sequence
  Amino acid sequence comprising a peptide comprising module 3 of CBD of MMP-9 with additional residues
STVMGGNSAGELCVFPFTFLGKEYSTCTSEGRGDGRLWCATTSNFDSDKKWGFCPDQG

SEQ ID NO: 31 - protein, 176 aa, Artificial Sequence
  Amino acid sequence comprising CBD of MMP-9 with additional residues
PTRFGNADGAACHFPFIFEGRSYSACTTDGRSDGLPWCSTTANYDTDDRFGFCPSERLYTQDGNADGKPCQFPFIFQGQSYSACTTDGRSDGYRWCATTANYDRDKLFGFCPTRADSTVMGGNSAGELCVFPFTFLGKEYSTCTSEGRGDGRLWCATTSNFDSDKKWGFCPDQGYS

SEQ ID NO: 32 - protein, 6 aa, Artificial Sequence
  Linker sequence 4
DQGYSL

SEQ ID NO: 33 - protein, 707 aa, Homo sapiens
MSLWQPLVLVLLVLGCCFAAPRQRQSTLVLFPGDLRTNLTDRQLAEEYLYRYGYTRVAEMRGESKSLGPALLLLQKQLSLPETGELDSATLKAMRTPRCGVPDLGRFQTFEGDLKWHHHNITYWIQNYSEDLPRAVIDDAFARAFALWSAVTPLTFTRVYSRDADIVIQFGVAEHGDGYPFDGKDGLLAHAFPPGPGIQGDAHFDDDELWSLGKGVVVPTRFGNADGAACHFPFIFEGRSYSACTTDGRSDGLPWCSTTANYDTDDRFGFCPSERLYTQDGNADGKPCQFPFIFQGQSYSACTTDGRSDGYRWCATTANYDRDKLFGFCPTRADSTVMGGNSAGELCVFPFTFLGKEYSTCTSEGRGDGRLWCATTSNFDSDKKWGFCPDQGYSLFLVAAHEFGHALGLDHSSVPEALMYPMYRFTEGPPLHKDDVNGIRHLYGPRPEPEPRPPTTTTPQPTAPPTVCPTGPPTVHPSERPTAGPTGPPSAGPTGPPTAGPSTATTVPLSPVDDACNVNIFDAIAEIGNQLYLFKDGKYWRFSEGRGSRPQGPFLIADKWPALPRKLDSVFEERLSKKLFFFSGRQVWVYTGASVLGPRRLDKLGLGADVAQVTGALRSGRGKMLLFSGRRLWRFDVKAQMVDPRSASEVDRMFPGVPLDTHDVFQYREKAYFCQDRFYWRVSSRSELNQVDQVGYVTYDILQCPED

SEQ ID NO: 34 - protein, 49 aa, Homo sapiens
ADGAACHFPFIFEGRSYSACTTDGRSDGLPWCSTTANYDTDDRFGFCPS

SEQ ID NO: 35 - protein, 60 aa, Artificial Sequence
  Amino acid sequence of a peptide comprising module 1 of CBD of MMP-9 with additional residues
TRFGNADGAACHFPFIFEGRSYSACTTDGRSDGLPWCSTTANYDTDDRFGFCPSERLYTQ

SEQ ID NO: 36 - protein, 49 aa, Homo sapiens
ADGKPCQFPFIFQGQSYSACTTDGRSDGYRWCATTANYDRDKLFGFCPT

SEQ ID NO: 37 - protein, 59 aa, Artificial Sequence
  Amino acid sequence of a peptide comprising module 2 of CBD of MMP-9 with additional residues
RLYTQDGNADGKPCQFPFIFQGQSYSACTTDGRSDGYRWCATTANYDRDKLFGFCPTRA

SEQ ID NO: 38 - protein, 49 aa, Homo sapiens
SAGELCVFPFTFLGKEYSTCTSEGRGDGRLWCATTSNFDSDKKWGFCPD